European Patent Specification EP 3 619 321 B1, published July 17, 2024. Title: DP04 POLYMERASE VARIANTS. Applicant: Stratos Genomics Inc. Kokoris, Mark Stamatios Prindle, Marc Chase, Jack Busam, Robert Kovarik, Michael Keller, Salka Murt, Megan Thiessen, Greg. The sequence listing filed with the application follows.

SEQUENCE LISTING (106 sequences)

SEQ ID NO: 1 - protein, 352 aa, Sulfolobus solfataricus
MIVLFVDFDYFYAQVEEVLNPSLKGKPVVVCVFSGRFEDSGAVATANYEARKFGVKAGIPIVEAKKILPNAVYLPMRKEVYQQVSSRIMNLLREYSEKIEIASIDEAYLDISDKVRDYREAYNLGLEIKNKILEKEKITVTVGISKNKVFAKIAADMAKPNGIKVIDDEEVKRLIRELDIADVPGIGNITAEKLKKLGINKLVDTLSIEFDKLKGMIGEAKAKYLISLARDEYNEPIRTRVRKSIGRIVTMKRNSRNLEEIKPYLFRAIEESYYKLDKRIPKAIHVVAVTEDLDIVSRGRTFPHGISKETAYSESVKLLQKILEEDERKIRRIGVRFSKFIEAIGLDKFFDT

SEQ ID NO: 2 - protein, 340 aa, Sulfolobus solfataricus
MIVLFVDFDYFYAQVEEVLNPSLKGKPVVVCVFSGRFEDSGVVATANYEARKFGVYAGIPIVEAKKILPNAVYLPWRNLVYWGVSERIMNLLREYSEKIEIASIDEAYLDISDKVRDYREAYNLGLEIKNKILEKEKITVTVGISKNKVFAEMAGRMAKPNGIKVIDDEEVKRLIRELDIADVLGIPYWYAEKLKKLGINKLVDTLSIEFDKLKGMIGEAKAKYLISLARDEYNEPIRTRVRKSIGRTVTMKRNSRNLEEIKPYLFRAIEESYYKLDKRIPKAIHVVAWKSYWDIVSRGRTFPHGISKETAYSESVKLLQKILEEDERKIRRIGVRFSKF

SEQ ID NO: 3 - protein, 340 aa, Sulfolobus solfataricus
MIVLFVDFDYFYAQVEEVLNPSLKGKPVVVCVFSGRFEDSGVVATANYEARKFGVYAGIPIVEAKKILPNAVYLPWRNLVYWGVSERIMNLLREYSEKIEIASIDEAYLDISDKVRDYREAYNLGLEIKNKILEKEKITVTVGISKNKVFAGTAGLMAKPNGIKVIDDEEVKRLIRELDIADVLGIPYWYAEKLKKLGINKLVDTLSIEFDKLKGMIGEAKAKYLISLARDEYNEPIRTRVRKSIGRTVTMKRNSRNLEEIKPYLFRAIEESYYKLDKRIPKAIHVVAWKSYWDIVSRGRTFPHGISKETAYSESVKLLQKILEEDERKIRRIGVRFSKF

SEQ ID NO: 4 - protein, 340 aa, Sulfolobus solfataricus
MIVLFVDFDYFYAQVEEVLNPSLKGKPVVVCVFSGRFEDSGVVATANYEARKFGVYAGIPIVEAKKILPNAVYLPWRNLVYWGVSERIMNLLREYSEKIEIASIDEAYLDISDKVRDYREAYNLGLEIKNKILEKEKITVTVGISKNKVFALTAGRMAKPNGIKVIDDEEVKRLIRELDIADVLGIPYWYAEKLKKLGINKLVDTLSIEFDKLKGMIGEAKAKYLISLARDEYNEPIRTRVRKSIGRTVTMKRNSRNLEEIKPYLFRAIEESYYKLDKRIPKAIHVVAWKSYWDIVSRGRTFPHGISKETAYSESVKLLQKILEEDERKIRRIGVRFSKF

SEQ ID NO: 5 - protein, 340 aa, Sulfolobus solfataricus
MIVLFVDFDYFYAQVEEVLNPSLKGKPVVVCVFSGRFEDSGVVATANYEARKFGVYPGIPIVEAKKILPNAVYLPWRNLVYWGVSEQIMNLLREYSEKIEIASIDEAYLDISDKVRDYREAYNLGLEIKNKILEKEKITVTVGISKNKVFAGIAMWMAKPNGIKVIDDEEVKRLIRELDIADVLGIGNWTAEKLKSLGINKLVDTLSIEFDKLKGMIGEAKAKYLISLARDEYNEPIRTRVRKSIGRTVTMKNNSTNLEEIKPYLFRAIEESYYKLDNQIPKAIHVVAWRSYWDYVHRLRRFPHGISKETAYSESVKLLQKILEEDERKIRRIGVRFSKF

SEQ ID NO: 6 - protein, 340 aa, Sulfolobus solfataricus
MIVLFVDFDYFYAQVEEVLNPSLKGKPVVVCVFSGRFEDSGVVATANYEARKFGVYPGIPIVEAKKILPNAVYLPWRNLVYWGVSERIMNLLREYSEKIEIASIDEAYLDISDKVNDYREAYNLGLEIKNKILEKEKITVTVGISKNKVFAGIAMWMAKPNGIKVIDDEEVKNLINELDIADVLGIGNWTAEKLKKLGINKLVDTLSIEFDKLKGMIGEAKAKYLISLARDEYNEPIRTRVRKSIGRTVTMKRNSRNLEEIKPYLFRAIEESYYKLDKRIPKAIHVVAWRSYWDYVHRLRRFPHGISKETAYSESVQLLQKILEEDERKIRRIGVRFSKF

SEQ ID NO: 7 - protein, 340 aa, Sulfolobus solfataricus
MIVLFVDFDYFYAQVEEVLNPSLKGKPVVVCVFSGRFEDSGVVATANYEARKFGVYPGIPIVEAKKILPNAVYLPWRNLVYWGVSERIMNLLREYSEKIEIASIDEAYLDISDKVRDYREAYNLGLEIKNKILEKEKITVTVGISKNKVFAGIAMWMAKPNGIKVIDDEEVKRLIRELDIADVLGIGNWTAEKLKKLGINKLVDTLSIEFDKLKGMIGEAKAKYLISLARDEYNEPIRTRVRKSIGRTVTMKRNSRNLEEIKPYLFRAIEESYYKLDKRIPKAIHVVAWRSYWDYVHRLRRFPHGISKETAYSESVKLLQKILKEDKRKIRRIGVRFSKF

SEQ ID NO: 8 - protein, 340 aa, Sulfolobus solfataricus
MIVLFVDFDYFYAQVEEVLNPSLKGKPVVVCVFSGRFEDSGVVATANYEARKFGVYPGIPIVEAKKILPNAVYLPWRNLVYWGVSERIMNLLREYSEKIEIASIDEAYLDISDKVNDYREAYNLGLEIKNKILEKEKITVTVGISKNKVFAGIAMWMAKPNGIKVIDDEEVKNLINELDIADVLGIGNWTAEKLKKLGINKLVDTLSIEFDKLKGMIGEAKAKYLISLARDEYNEPIRTRVRKSIGRTVTMKRNSRNLEEIKPYLFRAIEESYYKLDKRIPKAIHVVAWRSYWDYVHRLRRFPHGISKETAYSESVKLLQKILKEDKRKIRRIGVRFSKF

SEQ ID NO: 9 - protein, 340 aa, Sulfolobus solfataricus
MIVLFVDFDYFYAQVEEVLNPSLKGKPVVVCVFSGRFEDSGVVATANYEARKFGVYPGIPIVEAKKILPNAVYLPWRNLVYWGVSERIMNLLREYSEKIEIASIDEAYLDISDKVRDYREAYNLGLEIKNKILEKEKITVTVGISKNKVFAGIAMWMAKPNGITVIDDEEVKRLIRELDIADVLGIGNWTAEKLKKLGINKLVDTLSIEFDKLKGMIGEAKAKYLISLARDEYNEPIRTRVRKSIGRTVTMKRNSRNLEEIKPYLFRAIEESYYKLDKRIPKAIHVVAWRSYWDYVHRLRRFPHGISKETAYSESVKLLQKILEEDERKIRRIGVRFSKF

SEQ ID NO: 10 - protein, 340 aa, Sulfolobus solfataricus
MIVLFVDFDYFYAQVEEVLNPSLKGKPVVVCVFSGRFEDSGVVATANYEARKFGVYPGIPIVEAKKILPNAVYLPWRNLVYWGVSERIMNLLREYSEKIEIASIDEAYLDISDKVRDYREAYNLGLEIKNKILEKEKITVTVGISKNKVFAGIAMWMAKPNGIKVIDDEEVKRLIRELDIADVLGIGNWTARKLKLLGINKLVDTLSIEFDKLKGMIGEAKAKYLISLARDEYNEPIRTRVWKSIGRTVTMKRNSRNLEEIKPYLFRAIEESYYKLDKRIPGAIHVVAWRSYWDYVHRLRRFPHGISKETAYSESVKLLQKILEEDERKIRRIGVRFSKF

SEQ ID NO: 11 - protein, 340 aa, Sulfolobus solfataricus
MIVLFVDFDYFYAQVEEVLNPSLKGKPVVVCVFSGRFEDSGVVATANYEARKFGVYPGIPIVEAKKILPNAVYLPWRNLVYWGVSERIMNLLREYSEKIEIASIDEAYLDISDKVNDYREAYNLGLEIKNKILEKEKITVTVGISKNKVFAGIAMWMAKPNGIKVIDDEEVKNLINELDIADVLGIGNWTAEKLKKLGINKLVDTLSIEFDKLKGMIGEAKAKYLISLARDEYNEPIRTRVRKSIGRTVTMKRNSRNLEEIKPYLFRAIEESYYKLDKRIPKAIHVVAWRSYWDYVHRLRRFPHGISKETAYSESVQLLQQILKKDKRKIRRIGVRFSKF

SEQ ID NO: 12 - protein, 340 aa, Sulfolobus solfataricus
MIVLFVDFDYFYAQVEEVLNPSLKGKPVVVCVFSGRFEDSGVVATANYEARKFGVYPGIPIVEAKKILPNAVYLPWRNLVYWGVSERIMNLLREYSEKIEIASIDEAYLDISDKVNDYREAYNLGLEIKNKILEKEKITVTVGISKNKVFAGIAMWMAKPNGIKVIDDEEVKNLINELDIADVLGIGNWTAEKLKKLGINKLVDTLSIEFDKLKGMIGEAKAKYLISLARDEYNEPIRTRVRKSIGRTVTMKRNSRNLEEIKPYLFRAIEESYYKLDKRIPKAIHVVAWRSYWDYVHRLRRFPHGISKETAYSESVQLLQQILNQDQRKIRRIGVRFSKF

SEQ ID NO: 13 - protein, 340 aa, Sulfolobus solfataricus
MIVLFVDFDYFYAQVEEVLNPSLKGKPVVVCVFSGRFEDSGVVATANYEARKFGVYAGIPIVEAKKILPNAVYLPWRNLVYWGVSERIMNLLREYSEKIEIASIDEAYLDISDKVRDYREAYNLGLEIKNKILEKEKITVTVGISKNKVFAGTAGLMAKPNGIKVIDDEEVKRLIRELDIADVLGIGNWTAEKLKKLGINKLVDTLSIEFDKLKGMIGEAKAKYLISLARDEYNEPIRTRVRKSIGRIVTMKRNSRNLEEIKPYLFRAIEESYYKLDKRIPKAIHVVAWKSYWDIVSRGRTFPHGISKETAYSESVKLLQKILKEDKRKIRRIGVRFSKF

SEQ ID NO: 14 - protein, 340 aa, Sulfolobus solfataricus
MIVLFVDFDYFYAQVEEVLNPSLKGKPVVVCVFSGRFEDSGVVATANYEARKFGVYAGIPIVEAKKILPNAVYLPWRNLVYWGVSERIMNLLREYSEKIEIASIDEAYLDISDKVRDYREAYNLGLEIKNKILEKEKITVTVGISKNKVFAGIAMWMAKPNGIKVIDDEEVKRLIRELDIADVLGIPYWYAEKLKKLGINKLVDTLSIEFDKLKGMIGEAKAKYLISLARDEYNEPIRTRVRKSIGRTVTMKRNSRNLEEIKPYLFRAIEESYYKLDKRIPKAIHVVAWKSYWDIVSRGRTFPHGISKETAYSESVKLLQKILKEDKRKIRRIGVRFSKF

SEQ ID NO: 15 - protein, 340 aa, Sulfolobus solfataricus
MIVLFVDFDYFYAQVEEVLNPSLKGKPVVVCVFSGRFEDSGVVATANYEARKFGVYPGIPIVEAKKILPNAVYLPWRNLVYWGVSERIMNLLREYSEKIEIASIDEAYLDISDKVRDYREAYNLGLEIKNKILEKEKITVTVGISKNKVFAGIAMWMAKPNGIKVIDDEEVKRLIRELDIADVLGIGNWTARKLKLLGINKLVDTLSIEFDKLKGMIGEAKAKYLISLARDEYNEPIRTRVWKSIGRTVTMKRNSRNLEEIKPYLFRAIEESYYKLDKRIPGAIHVVAWRSYWDYVHRLRRFPHGISKETAYSESVKLLQKILREDRRKIRRIGVRFSKF

SEQ ID NO: 16 - protein, 340 aa, Sulfolobus solfataricus
MIVLFVDFDYFYAQVEEVLNPSLKGKPVVVCVFSGRFEDSGVVATANYEARKFGVYAGIPIVEAKKILPNAVYLPWRNLVYWGVSERIMNLLREYSEKIEIASIDEAYLDISDKVRDYREAYNLGLEIKNKILEKEKITVTVGISKNKVFAGTAGLMAKPNGIKVIDDEEVKRLIRELDIADVLGIGNWTAEKLKKLGINKLVDTLSIEFDKLKGMIGEAKAKYLISLARDEYNEPIRTRVRKSIGRIVTMKRNSRNLEEIKPYLFRAIEESYYKLDKRIPKAIHVVAWKSYWDIVSRGRTFPHGISKETAYSESVQLLQQILKKDKRKIRRIGVRFSKF

SEQ ID NO: 17 - protein, 340 aa, Sulfolobus solfataricus
MIVLFVDFDYFYAQVEEVLNPSLKGKPVVVCVFSGRFEDSGVVATANYEARKFGVYAGIPIVEAKKILPNAVYLPWRNLVYWGVSERIMNLLREYSEKIEIASIDEAYLDISDKVRDYREAYNLGLEIKNKILEKEKITVTVGISKNKVFAGIAMWMAKPNGIKVIDDEEVKRLIRELDIADVLGIPYWYAEKLKKLGINKLVDTLSIEFDKLKGMIGEAKAKYLISLARDEYNEPIRTRVRKSIGRTVTMKRNSRNLEEIKPYLFRAIEESYYKLDKRIPKAIHVVAWKSYWDIVSRGRTFPHGISKETAYSESVQLLQQILKKDKRKIRRIGVRFSKF

SEQ ID NO: 18 - protein, 340 aa, Sulfolobus solfataricus
MIVLFVDFDYFYAQVEEVLNPSLKGKPVVVCVFSGRFEDSGVVATANYEARKFGVYAGIPIVEAKKILPNAVYLPWRNLVYWGVSERIMNLLREYSEKIEIASIDEAYLDISDKVRDYREAYNLGLEIKNKILEKEKITVTVGISKNKVFAGIAMWMAKPNGIKVIDDEEVKRLIRELDIADVLGIPYWYAEKLKKLGINKLVDTLSIEFDKLKGMIGEAKAKYLISLARDEYNEPIRTRVRKSIGRTVTMKRNSRNLEEIKPYLFRAIEESYYKLDKRIPKAIHVVAWKSYWDIVSRGRTFPHGISKETAYSESVQLLQQILNQDQRKIRRIGVRFSKF

SEQ ID NO: 19 - protein, 340 aa, Sulfolobus solfataricus
MIVLFVDFDYFYAQVEEVLNPSLKGKPVVVCVFSGRFEDSGVVATANYEARKFGVYAGIPIVEAKKILPNAVYLPWRNLVYWGVSERIMNLLREYSEKIEIASIDEAYLDISDKVRDYREAYNLGLEIKNKILEKEKITVTVGISKNKVFAGTAGLMAKPNGIKVIDDEEVKRLIRELDIADVLGIGNWTAEKLKKLGINKLVDTLSIEFDKLKGMIGEAKAKYLISLARDEYNEPIRTRVRKSIGRIVTMKRNSRNLEEIKPYLFRAIEESYYKLDKRIPKAIHVVAWKSYWDIVSRGRTFPHGISKETAYSESVKLLQKILEKKERKIRRIGVRFSKF

SEQ ID NO: 20 - protein, 340 aa, Sulfolobus solfataricus
MIVLFVDFDYFYAQVEEVLNPSLKGKPVVVCVFSGRFEDSGVVATANYEARKFGVYAGIPIVEAKKILPNAVYLPWRNLVYWGVSERIMNLLREYSEKIEIASIDEAYLDISDKVRDYREAYNLGLEIKNKILEKEKITVTVGISKNKVFAQRAGAMAKPNGIKVIDDEEVKRLIRELDIADVLGIPYWYAEKLKKLGINKLVDTLSIEFDKLKGMIGEAKAKYLISLARDEYNEPIRTRVRKSIGRTVTMKRNSRNLEEIKPYLFRAIEESYYKLDKRIPKAIHVVAWKSYWDIVSRGRTFPHGISKETAYSESVKLLQKILEEDERKIRRIGVRFSKF

SEQ ID NO: 21 - protein, 340 aa, Sulfolobus solfataricus
MIVLFVDFDYFYAQVEEVLNPSLKGKPVVVCVFSGRFEDSGVVATANYEARKFGVYAGIPIVEAKKILPNAVYLPWRNLVYWGVSERIMNLLREYSEKIEIASIDEAYLDISDKVRDYREAYNLGLEIKNKILEKEKITVTVGISKNKVFAGIAMWMAKPNGIKVIDDEEVKRLIRELDIADVLGIGNWTAEKLKKLGINKLVDTLSIEFDKLKGMIGEAKAKYLISLARDEYNEPIRTRVRKSIGRTVTMKRNSRNLEEIKPYLFRAIEESYYKLDKRIPKAIHVVAWRSYWQMATLFRHFPHGISKETAYSESVKLLQKILEEDERKIRRIGVRFSKF

SEQ ID NO: 22 - protein, 340 aa, Sulfolobus solfataricus
MIVLFVDFDYFYAQVEEVLNPSLKGKPVVVCVFSGRFEDSGVVATANYEARKFGVYAGIPIVEAKKILPNAVYLPWRNLVYWGVSERIMNLLREYSEKIEIASIDEAYLDISDKVRDYREAYNLGLEIKNKILEKEKITVTVGISKNKVFAGIAMWMAKPNGIKVIDDEEVKRLIRELDIADVLGIGNWTAEKLKKLGINKLVDTLSIEFDKLKGMIGEAKAKYLISLARDEYNEPIRTRVRKSIGRTVTMKRNSRNLEEIKPYLFRAIEESYYKLDKRIPKAIHVVAWRSYWDAVPRWRFFPHGISKETAYSESVKLLQKILEEDERKIRRIGVRFSKF

SEQ ID NO: 23 - protein, 340 aa, Sulfolobus solfataricus
MIVLFVDFDYFYAQVEEVLNPSLKGKPVVVCVFSGRFEDSGVVATANYEARKFGVYAGIPIVEAKKILPNAVYLPWRNLVYWGVSERIMNLLREYSEKIEIASIDEAYLDISDKVRDYREAYNLGLEIKNKILEKEKITVTVGISKNKVFAGIAMWMAKPNGIKVIDDEEVKRLIRELDIADVLGIGNWTAEKLKKLGINKLVDTLSIEFDKLKGMIGEAKAKYLISLARDEYNEPIRTRVRKSIGRTVTMKRNSRNLEEIKPYLFRAIEESYYKLDKRIPKAIHVVAWRSYWDYVWRWRVFPHGISKETAYSESVKLLQKILEEDERKIRRIGVRFSKF

SEQ ID NO: 24 - protein, 340 aa, Sulfolobus solfataricus
MIVLFVDFDYFYAQVEEVLNPSLKGKPVVVCVFSGRFEDSGVVATANYEARKFGVYAGIPIVEAKKILPNAVYLPWRNLVYWGVSERIMNLLREYSEKIEIASIDEAYLDISDKVRDYREAYNLGLEIKNKILEKEKITVTVGISKNKVFAGIAMWMAKPNGIKVIDDEEVKRLIRELDIADVLGIGNWTAEKLKKLGINKLVDTLSIEFDKLKGMIGEAKAKYLISLARDEYNEPIRTRVRKSIGRTVTMKRNSRNLEEIKPYLFRAIEESYYKLDKRIPKAIHVVAWRSYWDCVWRIRWFPHGISKETAYSESVKLLQKILEEDERKIRRIGVRFSKF

SEQ ID NO: 25 - protein, 340 aa, Sulfolobus solfataricus
MIVLFVDFDYFYAQVEEVLNPSLKGKPVVVCVFSGRFEDSGVVATANYEARKFGVYAGIPIVEAKKILPNAVYLPWRNLVYWGVSERIMNLLREYSEKIEIASIDEAYLDISDKVRDYREAYNLGLEIKNKILEKEKITVTVGISKNKVFAGIAMWMAKPNGIKVIDDEEVKRLIRELDIADVLGIGNWTAEKLKKLGINKLVDTLSIEFDKLKGMIGEAKAKYLISLARDEYNEPIRTRVRKSIGRTVTMKRNSRNLEEIKPYLFRAIEESYYKLDKRIPGLIHVVAWKSYWDIVSRGRTERGGISKETAYSESVKLLQKILEEDERKIRRIGVRFSKF

SEQ ID NO: 26 - protein, 340 aa, Sulfolobus solfataricus
MIVLFVDFDYFYAQVEEVLNPSLKGKPVVVCVFSGRFEDSGVVATANYEARKFGVYAGIPIVEAKKILPNAVYLPWRNLVYWGVSERIMNLLREYSEKIEIASIDEAYLDISDKVRDYREAYNLGLEIKNKILEKEKITVTVGISKNKVFAGHAGRMAKPNGIKVIDDEEVKRLIRELDIADVLGIPYWYAEKLKKLGINKLVDTLSIEFDKLKGMIGEAKAKYLISLARDEYNEPIRTRVRKSIGRTVTMKRNSRNLEEIKPYLFRAIEESYYKLDKRIPKAIHVVAWKSYWDIVSRGRTFPHGISKETAYSESVKLLQKILEEDERKIRRIGVRFSKF

SEQ ID NO: 27 - protein, 340 aa, Sulfolobus solfataricus
MIVLFVDFDYFYAQVEEVLNPSLKGKPVVVCVFSGRFEDSGVVATANYEARKFGVYAGIPIVEAKKILPNAVYLPWRNLVYWGVSERIMNLLREYSEKIEIASIDEAYLDISDKVRDYREAYNLGLEIKNKILEKEKITVTVGISKNKVFAGIAMWMAKPNGIKVIDDEEVKRLIRELDIADVLGIGNWTAEKLKKLGINKLVDTLSIEFDKLKGMIGEAKAKYLISLARDEYNEPIRTRVRKSIGRTVTMKRNSRNLEEIKPYLFRAIEESYYKLDKRIPKAIHVVAWRSYWAPRLKACEFPHGISKETAYSESVKLLQKILEEDERKIRRIGVRFSKF

SEQ ID NO: 28 - protein, 340 aa, Sulfolobus solfataricus
MIVLFVDFDYFYAQVEEVLNPSLKGKPVVVCVFSGRFEDSGVVATANYEARKFGVYAGIPIVEAKKILPNAVYLPWRNLVYWGVSERIMNLLREYSEKIEIASIDEAYLDISDKVRDYREAYNLGLEIKNKILEKEKITVTVGISKNKVFAGIAMWMAKPNGIKVIDDEEVKRLIRELDIADVLGIGNWTAEKLKKLGINKLVDTLSIEFDKLKGMIGEAKAKYLISLARDEYNEPIRTRVRKSIGRTVTMKRNSRNLEEIKPYLFRAIEESYYKLDKRIPKAIHVVAWRSYWCISQTGRLFPHGISKETAYSESVKLLQKILEEDERKIRRIGVRFSKF

SEQ ID NO: 29 - protein, 340 aa, Sulfolobus solfataricus
MIVLFVDFDYFYAQVEEVLNPSLKGKPVVVCVFSGRFEDSGVVATANYEARKFGVYAGIPIVEAKKILPNAVYLPWRNLVYWGVSERIMNLLREYSEKIEIASIDEAYLDISDKVRDYREAYNLGLEIKNKILEKEKITVTVGISKNKVFAGIAMWMAKPNGIKVIDDEEVKRLIRELDIADVLGIGNWTAEKLKKLGINKLVDTLSIEFDKLKGMIGEAKAKYLISLARDEYNEPIRTRVRKSIGRTVTMKRNSRNLEEIKPYLFRAIEESYYKLDKRIPKAIHVVAWRSYWSTRSTHSYFPHGISKETAYSESVKLLQKILEEDERKIRRIGVRFSKF

SEQ ID NO: 30 - protein, 340 aa, Sulfolobus solfataricus
MIVLFVDFDYFYAQVEEVLNPSLKGKPVVVCVFSGRFEDSGVVATANYEARKFGVYAGIPIVEAKKILPNAVYLPWRNLVYWGVSERIMNLLREYSEKIEIASIDEAYLDISDKVRDYREAYNLGLEIKNKILEKEKITVTVGISKNKVFAGIAMWMAKPNGIKVIDDEEVKRLIRELDIADVLGIGNWTAEKLKKLGINKLVDTLSIEFDKLKGMIGEAKAKYLISLARDEYNEPIRTRVRKSIGRTVTMKRNSRNLEEIKPYLFRAIEESYYKLDKRIPKAIHVVAWRSYWNSQYRWSWFPHGISKETAYSESVKLLQKILEEDERKIRRIGVRFSKF

SEQ ID NO: 31 - protein, 340 aa, Sulfolobus solfataricus
MIVLFVDFDYFYAQVEEVLNPSLKGKPVVVCVFSGRFEDSGVVATANYEARKFGVYAGIPIVEAKKILPNAVYLPWRNLVYWGVSERIMNLLREYSEKIEIASIDEAYLDISDKVRDYREAYNLGLEIKNKILEKEKITVTVGISKNKVFAGIAMWMAKPNGIKVIDDEEVKRLIRELDIADVLGIGNWTAEKLKKLGINKLVDTLSIEFDKLKGMIGEAKAKYLISLARDEYNEPIRTRVRKSIGRTVTMKRNSRNLEEIKPYLFRAIEESYYKLDKRIPKAIHVVAWRSYWLTRCRGRRFPHGISKETAYSESVKLLQKILEEDERKIRRIGVRFSKF

SEQ ID NO: 32 - protein, 340 aa, Sulfolobus solfataricus
MIVLFVDFDYFYAQVEEVLNPSLKGKPVVVCVFSGRFEDSGVVATANYEARKFGVYAGIPIVEAKKILPNAVYLPWRNLVYWGVSERIMNLLREYSEKIEIASIDEAYLDISDKVRDYREAYNLGLEIKNKILEKEKITVTVGISKNKVFAGIAMWMAKPNGIKVIDDEEVKRLIRELDIADVLGIGNWTAEKLKKLGINKLVDTLSIEFDKLKGMIGEAKAKYLISLARDEYNEPIRTRVRKSIGRTVTMKRNSRNLEEIKPYLFRAIEESYYKLDKRIPKAIHVVAWRSYWAWRRESSMFPHGISKETAYSESVKLLQKILEEDERKIRRIGVRFSKF

SEQ ID NO: 33 - protein, 340 aa, Sulfolobus solfataricus
MIVLFVDFDYFYAQVEEVLNPSLKGKPVVVCVFSGRFEDSGVVATANYEARKFGVYAGIPIVEAKKILPNAVYLPWRNLVYWGVSERIMNLLREYSEKIEIASIDEAYLDISDKVRDYREAYNLGLEIKNKILEKEKITVTVGISKNKVFAARAGLMAKPNGIKVIDDEEVKRLIRELDIADVLGIPYWYAEKLKKLGINKLVDTLSIEFDKLKGMIGEAKAKYLISLARDEYNEPIRTRVRKSIGRTVTMKRNSRNLEEIKPYLFRAIEESYYKLDKRIPKAIHVVAWKSYWDIVSRGRTFPHGISKETAYSESVKLLQKILEEDERKIRRIGVRFSKF

SEQ ID NO: 34 - protein, 340 aa, Sulfolobus solfataricus
MIVLFVDFDYFYAQVEEVLNPSLKGKPVVVCVFSGRFEDSGVVATANYEARKFGVYAGIPIVEAKKILPNAVYLPWRNLVYWGVSERIMNLLREYSEKIEIASIDEAYLDISDKVRDYREAYNLGLEIKNKILEKEKITVTVGISKNKVFAGIAMWMAKPNGIKVIDDEEVKRLIRELDIADVLGIGNWTAEKLKKLGINKLVDTLSIEFDKLKGMIGEAKAKYLISLARDEYNEPIRTRVRKSIGRTVTMKRNSRNLEEIKPYLFRAIEESYYKLDKRIPKAIHVVAWRSYWPPRSRACKFPHGISKETAYSESVKLLQKILEEDERKIRRIGVRFSKF

SEQ ID NO: 35 - protein, 340 aa, Sulfolobus solfataricus
MIVLFVDFDYFYAQVEEVLNPSLKGKPVVVCVFSGRFEDSGVVATANYEARKFGVYAGIPIVEAKKILPNAVYLPWRNLVYWGVSERIMNLLREYSEKIEIASIDEAYLDISDKVRDYREAYNLGLEIKNKILEKEKITVTVGISKNKVFAYSACGMAKPNGIKVIDDEEVKRLIRELDIADVLGIPYWYAEKLKKLGINKLVDTLSIEFDKLKGMIGEAKAKYLISLARDEYNEPIRTRVRKSIGRTVTMKRNSRNLEEIKPYLFRAIEESYYKLDKRIPKAIHVVAWKSYWDIVSRGRTFPHGISKETAYSESVKLLQKILEEDERKIRRIGVRFSKF

SEQ ID NO: 36 - protein, 340 aa, Sulfolobus solfataricus
MIVLFVDFDYFYAQVEEVLNPSLKGKPVVVCVFSGRFEDSGVVATANYEARKFGVYAGIPIVEAKKILPNAVYLPWRNLVYWGVSERIMNLLREYSEKIEIASIDEAYLDISDKVRDYREAYNLGLEIKNKILEKEKITVTVGISKNKVFAVYACGMAKPNGIKVIDDEEVKRLIRELDIADVLGIPYWYAEKLKKLGINKLVDTLSIEFDKLKGMIGEAKAKYLISLARDEYNEPIRTRVRKSIGRTVTMKRNSRNLEEIKPYLFRAIEESYYKLDKRIPKAIHVVAWKSYWDIVSRGRTFPHGISKETAYSESVKLLQKILEEDERKIRRIGVRFSKF

SEQ ID NO: 37 - protein, 340 aa, Sulfolobus solfataricus
MIVLFVDFDYFYAQVEEVLNPSLKGKPVVVCVFSGRFEDSGVVATANYEARKFGVYAGIPIVEAKKILPNAVYLPWRNLVYWGVSERIMNLLREYSEKIEIASIDEAYLDISDKVRDYREAYNLGLEIKNKILEKEKITVTVGISKNKVFAMQAGYMAKPNGIKVIDDEEVKRLIRELDIADVLGIPYWYAEKLKKLGINKLVDTLSIEFDKLKGMIGEAKAKYLISLARDEYNEPIRTRVRKSIGRTVTMKRNSRNLEEIKPYLFRAIEESYYKLDKRIPKAIHVVAWKSYWDIVSRGRTFPHGISKETAYSESVKLLQKILEEDERKIRRIGVRFSKF

SEQ ID NO: 38 - protein, 340 aa, Sulfolobus solfataricus
MIVLFVDFDYFYAQVEEVLNPSLKGKPVVVCVFSGRFEDSGVVATANYEARKFGVYAGIPIVEAKKILPNAVYLPWRNLVYWGVSERIMNLLREYSEKIEIASIDEAYLDISDKVRDYREAYNLGLEIKNKILEKEKITVTVGISKNKVFALKAGSMAKPNGIKVIDDEEVKRLIRELDIADVLGIPYWYAEKLKKLGINKLVDTLSIEFDKLKGMIGEAKAKYLISLARDEYNEPIRTRVRKSIGRTVTMKRNSRNLEEIKPYLFRAIEESYYKLDKRIPKAIHVVAWKSYWDIVSRGRTFPHGISKETAYSESVKLLQKILEEDERKIRRIGVRFSKF

SEQ ID NO: 39 - protein, 340 aa, Sulfolobus solfataricus
MIVLFVDFDYFYAQVEEVLNPSLKGKPVVVCVFSGRFEDSGVVATANYEARKFGVYAGIPIVEAKKILPNAVYLPWRNLVYWGVSERIMNLLREYSEKIEIASIDEAYLDISDKVRDYREAYNLGLEIKNKILEKEKITVTVGISKNKVFAGIAMWMAKPNGIKVIDDEEVKRLIRELDIADVLGIGNWTAEKLKKLGINKLVDTLSIEFDKLKGMIGEAKAKYLISLARDEYNEPIRTRVRKSIGRTVTMKRNSRNLEEIKPYLFRAIEESYYKLDKRIPKAIHVVAWRSYWDYVFRYRSFPHGISKETAYSESVKLLQKILEEDERKIRRIGVRFSKF

SEQ ID NO: 40 - protein, 340 aa, Sulfolobus solfataricus
MIVLFVDFDYFYAQVEEVLNPSLKGKPVVVCVFSGRFEDSGVVATANYEARKFGVYPGIPIVEAKKILPNAVYLPWRNLVYWGVSERIMNLLREYSEKIEIASIDEAYLDISDKVRDYREAYNLGLEIKNKILEKEKITVTVGISKNKVFAGIAMWMAKPNGIKVIDDEEVKRLIRELDIADVLGIGNWTAEKLKKLGINKLVDTLSIEFDKLKGMIGEAKAKYLISLARDEYNEPIRTRVRKSIGRTVTMKRNSRNLEEIKPYLFRAIEESYYKLDKRIPKAIHVVAWRSYWHWYQRGRTFPHGISKETAYSESVKLLQKILEEDERKIRRIGVRFSKF

SEQ ID NO: 41 - protein, 340 aa, Sulfolobus solfataricus
MIVLFVDFDYFYAQVEEVLNPSLKGKPVVVCVFSGRFEDSGVVATANYEARKFGVYAGIPIVEAKKILPNAVYLPWRNLVYWGVSERIMNLLREYSEKIEIASIDEAYLDISDKVRDYREAYNLGLEIKNKILEKEKITVTVGISKNKVFAEVAGRMAKPNGIKVIDDEEVKRLIRELDIADVLGIGNWTAEKLKKLGINKLVDTLSIEFDKLKGMIGEAKAKYLISLARDEYNEPIRTRVRKSIGRTVTMKRNSRNLEEIKPYLFRAIEESYYKLDKRIPKAIHVVAWRSYWDYVHRLRRFPHGISKETAYSESVKLLQKILEEDERKIRRIGVRFSKF

SEQ ID NO: 42 - protein, 340 aa, Sulfolobus solfataricus
MIVLFVDFDYFYAQVEEVLNPSLKGKPVVVCVFSGRFEDSGVVATANYEARKFGVYAGIPIVEAKKILPNAVYLPWRNLVYWGVSERIMNLLREYSEKIEIASIDEAYLDISDKVRDYREAYNLGLEIKNKILEKEKITVTVGISKNKVFAGIAMWMAKPNGIKVIDDEEVKRLIRELDIADVLGIGNWTAEKLKKLGINKLVDTLSIEFDKLKGMIGEAKAKYLISLARDEYNEPIRTRVRKSIGRTVTMKRNSRNLEEIKPYLFRAIEESYYKLDKRIPKAIHVVAWRSYWSFATGGRQFPHGISKETAYSESVKLLQKILEEDERKIRRIGVRFSKF

SEQ ID NO: 43 - protein, 340 aa, Sulfolobus solfataricus
MIVLFVDFDYFYAQVEEVLNPSLKGKPVVVCVFSGRFEDSGVVATANYEARKFGVYAGIPIVEAKKILPNAVYLPWRNLVYWGVSERIMNLLREYSEKIEIASIDEAYLDISDKVRDYREAYNLGLEIKNKILEKEKITVTVGISKNKVFAGTAGLMAKPNGIKVIDDEEVKRLIRELDIADVLGIPYWYAEKLKKLGINKLVDTLSIEFDKLKGMIGEAKAKYLISLARDEYNEPIRTRVRKSIGRTVTMKRNSRNLEEIKPYLFRAIEESYYKLDKRIPKAIHVVAWKSYWDIVSRGRTFPHGISKETAYSESVKLLQKILKEDKRKIRRIGVRFSKF

SEQ ID NO: 44 - protein, 340 aa, Sulfolobus solfataricus
MIVLFVDFDYFYAQVEEVLNPSLKGKPVVVCVFSGRFEDSGVVATANYEARKFGVYAGIPIVEAKKILPNAVYLPWRNLVYWGVSERIMNLLREYSEKIEIASIDEAYLDISDKVRDYREAYNLGLEIKNKILEKEKITVTVGISKNKVFAGIAMWMAKPNGIKVIDDEEVKRLIRELDIADVLGIGNWTAEKLKKLGINKLVDTLSIEFDKLKGMIGEAKAKYLISLARDEYNEPIRTRVRKSIGRTVTMKRNSRNLEEIKPYLFRAIEESYYKLDKRIPKAIHVVAWRSYWPPVYLGVRFPHGISKETAYSESVKLLQKILEEDERKIRRIGVRFSKF

SEQ ID NO: 45 - protein, 340 aa, Sulfolobus solfataricus
MIVLFVDFDYFYAQVEEVLNPSLKGKPVVVCVFSGRFEDSGVVATANYEARKFGVYAGIPIVEAKKILPNAVYLPWSNLVYWGVSERIMNLLREYSSKIEIASIDEAYLDISDKVRDYREAYNLGLEIKNKILEKEKITVTVGISKNKVFAGTAGLMAKPNGIKVIDDEEVKRLIRELDIADVLGIPYWYAEKLKKLGINKLVDTLSIEFDKLKGMIGEAKAKYLISLARDEYNEPIRTRVRKSIGRTVTMKRNSRNLEEIKPYLFRAIEESYYKLDKRIPKAIHVVAWKSYWDIVSRGRTFPHGISKETAYSESVKLLQKILEEDERKIRRIGVRFSKF

SEQ ID NO: 46 - protein, 340 aa, Sulfolobus solfataricus
MIVLFVDFDYFYAQVEEVLNPSLKGKPVVVCVFSGRFEDSGVVATANYEARKFGVYAGIPIVEAKKILPNAVYLPWRNLVYWGVSERIMNLLREYSEKIEIASIDEAYLDISDKVRDYREAYNLGLEIKNKILEKEKITVTVGISKNKVFAGTAGLMAKPNGIKVIDDEEVKRLIRELDIADVLGIPYWYAEKLKKLGINKLVDTLSIEFDKLKGMIGEAKAKYLISLARDEYNEPIRTRVRKSIGRTVTMKRNSRNLEEIKPYLFRAIEESYYKLDKRIPKAIHVVAWKSYWDIVSEGRTFPHGISKETAYSESVKLLQNILEEDENKIRRIGVRFSKF

SEQ ID NO: 47 - protein, 340 aa, Sulfolobus solfataricus
MIVLFVDFDYFYAQVEEVLNPSLKGKPVVVCVFSGRFEDSGVVATANYEARKFGVYAGIPIVEAKKILPNAVYLPWRNLVYWGVSERIMNLLREYSEKIEIASIDEAYLDISDKVRDYREAYNLGLEIKNKILEKEKITVTVGISKNKVFALTAGRMAKPNGIKVIDDEEVKRLIRELDIADVLGIESWVAEKLKKLGINKLVDTLSIEFDKLKGMIGEAKAKYLISLARDEYNEPIRTRVRKSIGRTVTMKRNSRNLEEIKPYLFRAIEESYYKLDKRIPKAIHVVAWKSYWDIVSRGITFPHGISKETAYSESVKLLQKILEEDERKIRRIGVRFSKF

SEQ ID NO: 48 - protein, 340 aa, Sulfolobus solfataricus
MIVLFVDFDYFYAQVEEVLNPSLKGKPVVVCVFSGRFEDSGVVATANYEARKFGVYAGIPIVEAKKILPNAVYLPWRNLVYWGVSERIMNLLREYSEKIEIASIDEAYLDISDKVRDYREAYNLGLEIKNKILEKEKITVTVGISKNKVFAAKAAIMAKPNGIKVIDDEEVKRLIRELDIADVLGIPYWYAEKLKKLGINKLVDTLSIEFDKLKGMIGEAKAKYLISLARDEYNEPIRTRVRKSIGRTVTMKRNSRNLEEIKPYLFRAIEESYYKLDKRIPKAIHVVAWKSYWDIVSRGRTFPHGISKETAYSESVKLLQKILEEDERKIRRIGVRFSKF

SEQ ID NO: 49 - protein, 340 aa, Sulfolobus solfataricus
MIVLFVDFDYFYAQVEEVLNPSLKGKPVVVCVFSGRFEDSGVVATANYEARKFGVYAGIPIVEAKKILPNAVYLPWRNLVYWGVSERIMNLLREYSEKIEIASIDEAYLDISDKVRDYREAYNLGLEIKNKILEKEKITVTVGISKNKVFALQAGMMAKPNGIKVIDDEEVKRLIRELDIADVLGIESWVAEKLKKLGINKLVDTLSIEFDKLKGMIGEAKAKYLISLARDEYNEPIRTRVRKSIGRTVTMKRNSRNLEEIKPYLFRAIEESYYKLDKRIPKAIHVVAWKSYWDIVSRGRTFPHGISKETAYSESVKLLQKILEEDERKIRRIGVRFSKF

SEQ ID NO: 50 - protein, 340 aa, Sulfolobus solfataricus
MIVLFVDFDYFYAQVEEVLNPSLKGKPVVVCVFSGRFEDSGVVATANYEARKFGVYAGIPIVEAKKILPNAVYLPWRNLVYWGVSERIMNLLREYSEKIEIASIDEAYLDISDKVRDYREAYNLGLEIKNKILEKEKITVTVGISKNKVFAGTAGLMAKPNGIKVIDDEEVKRLIRELDIADVLGIPYWYAEKLKKLGINKLVDTLSIEFPKLVGMIGWAKACYLISLARDEYNEPIRTRVRKSIGRTVTMKRNSRNLEEIKPYLFRAIEESYYKLDKRIPKAIHVVAWKSYWDIVSRGRTFPHGISKETAYSESVKLLQKILEEDERKIRRIGVRFSKF

SEQ ID NO: 51 - protein, 340 aa, Sulfolobus solfataricus
MIVLFVDFDYFYAQVEEVLNPSLKGKPVVVCVFSGRFEDSGVVATANYEARKFGVYAGIPIVEAKKILPNAVYLPWRNLVYWGVSERIMNLLREYSEKIEIASIDEAYLDISDKVRDYREAYNLGLEIKNKILEKEKITVTVGISKNKVFAGTAGLMAKPNGIKVIDDEEVKRLIRELDIADVLGIPYWYAEKLKKLGINKLVDTLSIEFSKLSGMIGGAKAKYLISLARDEYNEPIRTRVRKSIGRTVTMKRNSRNLEEIKPYLFRAIEESYYKLDKRIPKAIHVVAWKSYWDIVSRGRTFPHGISKETAYSESVKLLQKILEEDERKIRRIGVRFSKF

SEQ ID NO: 52 - protein, 340 aa, Sulfolobus solfataricus
MIVLFVDFDYFYAQVEEVLNPSLKGKPVVVCVFSGRFEDSGVVATANYEARKFGVYAGIPIVEAKKILPNAVYLPWRNLVYWGVSERIMNLLREYSEKIEIASIDEAYLDISDKVRDYREAYNLGLEIKNKILEKEKITVTVGISKNKVFAGTAGLMAKPNGIKVIDDEEVKRLIRELDIADVLGIPYWYAEKLKKLGINKLVDTLSIEFPKLVGMIGAAKATYLISLARDEYNEPIRTRVRKSIGRTVTMKRNSRNLEEIKPYLFRAIEESYYKLDKRIPKAIHVVAWKSYWDIVSRGRTFPHGISKETAYSESVKLLQKILEEDERKIRRIGVRFSKF

SEQ ID NO: 53 - protein, 340 aa, Sulfolobus solfataricus
MIVLFVDFDYFYAQVEEVLNPSLKGKPVVVCVFSGRFEDSGVVATANYEARKFGVYAGIPIVEAKKILPNAVYLPWRNLVYWGVSERIMNLLREYSEKIEIASIDEAYLDISDKVRDYREAYNLGLEIKNKILEKEKITVTVGISKNKVFAGTAGLMAKPNGIKVIDDEEVKRLIRELDIADVLGIPYWYAEKLKKLGINKLVDTLSIEFPKLAGMIGAAKARYLISLARDEYNEPIRTRVRKSIGRTVTMKRNSRNLEEIKPYLFRAIEESYYKLDKRIPKAIHVVAWKSYWDIVSRGRTFPHGISKETAYSESVKLLQKILEEDERKIRRIGVRFSKF

SEQ ID NO: 54 - protein, 340 aa, Sulfolobus solfataricus
MIVLFVDFDYFYAQVEEVLNPSLKGKPVVVCVFSGRFEDSGVVATANYEARKFGVYAGIPIVEAKKILPNAVYLPWRNLVYWGVSERIMNLLREYSEKIEIASIDEAYLDISDKVRDYREAYNLGLEIKNKILEKEKITVTVGISKNKVFAGTAGLMAKPNGIKVIDDEEVKRLIRELDIADVLGIPYYFAEKLKKLGINKLVDTLSIEFDKLKGMIGEAKAKYLISLARDEYNEPIRTRVRKSIGRTVTMKRNSRNLEEIKPYLFRAIEESYYKLDKRIPKAIHVVAWKSYWDIVSRGRTFPHGISKETAYSESVKLLQKILEEDERKIRRIGVRFSKF

SEQ ID NO: 55 - protein, 340 aa, Sulfolobus solfataricus
MIVLFVDFDYFYAQVEEVLNPSLKGKPVVVCVFSGRFEDSGVVATANYEARKFGVYAGIPIVEAKKILPNAVYLPWRNLVYWGVSERIMNLLREYSEKIEIASIDEAYLDISDKVRDYREAYNLGLEIKNKILEKEKITVTVGISKNKVFAGTAGLMAKPNGIKVIDDEEVKRLIRELDIADVLGIPYWYAEKLKKLGINKLVDTLSIEFDKLKGMIGEAKAKYLISLARDEYNEPIRTRVRKSIGRTVTMKRNSRNLEEIKPYLFRAIEESYYKLDKRIPKAIHVVAWKSYWDIVSRGRTFPHGISKETAYSESVKLLKRALARDERKIRRIGVRFSKF

SEQ ID NO: 56 - protein, 340 aa, Sulfolobus solfataricus
MIVLFVDFDYFYAQVEEVLNPSLKGKPVVVCVFSGRFEDSGVVATANYEARKFGVYAGIPIVEAKKILPNAVYLPWRNLVYWGVSERIMNLLREYSEKIEIASIDEAYLDISDKVRDYREAYNLGLEIKNKILEKEKITVTVGISKNKVFAGTAGLMAKPNGIKVIDDEEVKRLIRELDIADVLGIPYWYAEKLKKLGINKLVDTLSIEFDKLKGMIGEAKAKYLISLARDEYNEPIRTRVRKSIGRTVTMKRNSRNLEEIKPYLFRAIEESYYKLDKRIPKAIHVVAWKSYWDIVSRGRTFPHGISKETAYSESVKLLRSLLGGDERKIRRIGVRFSKF

SEQ ID NO: 57 - protein, 340 aa, Sulfolobus solfataricus
MIVLFVDFDYFYAQVEEVLNPSLKGKPVVVCVFSGRFEDSGVVATANYEARKFGVYAGIPIVEAKKILPNAVYLPWRNLVYWGVSERIMNLLREYSEKIEIASIDEAYLDISDKVRDYREAYNLGLEIKNKILEKEKITVTVGISKNKVFAGTAGLMAKPNGIKVIDDEEVKRLIRELDIADVLGIPYWYAEKLKKLGINKLVDTLSIEFDKLKGMIGEAKAKYLISLARDEYNEPIRTRVRKSIGRTVTMKRNSRNLEEIKPYLFRAIEESYYKLDKRIPKAIHVVAWKSYWDIVSRGRTFPHGISKETAYSESVKLLQRCLSGDERKIRRIGVRFSKF

SEQ ID NO: 58 - protein, 340 aa, Sulfolobus solfataricus
MIVLFVDFDYFYAQVEEVLNPSLKGKPVVVCVFSGRFEDSGVVATANYEARKFGVYAGIPIVEAKKILPNAVYLPWRNLVYWGVSERIMNLLREYSEKIEIASIDEAYLDISDKVRDYREAYNLGLEIKNKILEKEKITVTVGISKNKVFAGTAGLMAKPNGIKVIDDEEVKRLIRELDIADVLGIPYWYAEKLKKLGINKLVDTLSIEFDKLSRMIGAARARYLISLARDEYNEPIRTRVRKSIGRTVTMKRNSRNLEEIKPYLFRAIEESYYKLDKRIPKAIHVVAWKSYWDIVSRGRTFPHGISKETAYSESVKLLQKILEEDERKIRRIGVRFSKF

SEQ ID NO: 59 - protein, 340 aa, Sulfolobus solfataricus
MIVLFVDFDYFYAQVEEVLNPSLKGKPVVVCVFSGRFEDSGVVATANYEARKFGVYAGIPIVEAKKILPNAVYLPWRNLVYWGVSERIMNLLREYSEKIEIASIDEAYLDISDKVRDYREAYNLGLEIKNKILEKEKITVTVGISKNKVFAGTAGLMAKPNGIKVIDDEEVKRLIRELDIADVLGIPYWYAEKLKKLGINKLVDTLSIEFDKLVSMIGRARAKYLISLARDEYNEPIRTRVRKSIGRTVTMKRNSRNLEEIKPYLFRAIEESYYKLDKRIPKAIHVVAWKSYWDIVSRGRTFPHGISKETAYSESVKLLQKILEEDERKIRRIGVRFSKF

SEQ ID NO: 60 - protein, 340 aa, Sulfolobus solfataricus
MIVLFVDFDYFYAQVEEVLNPSLKGKPVVVCVFSGRFEDSGVVATANYEARKFGVYAGIPIVEAKKILPNAVYLPWRNLVYWGVSERIMNLLREYSEKIEIASIDEAYLDISDKVRDYREAYNLGLEIKNKILEKEKITVTVGISKNKVFAGTAGLMAKPNGIKVIDDEMVKGFIRELDIADVLGIPYWYAEKLKKLGINKLVDTLSIEFDKLKGMIGEAKAKYLISLARDEYNEPIRTRVRKSIGRTVTMKRNSRNLEEIKPYLFRAIEESYYKLDKRIPKAIHVVAWKSYWDIVSRGRTFPHGISKETAYSESVKLLQKILEEDERKIRRIGVRFSKF

SEQ ID NO: 61 - protein, 340 aa, Sulfolobus solfataricus
MIVLFVDFDYFYAQVEEVLNPSLKGKPVVVCVFSGRFEDSGVVATANYEARKFGVYAGIPIVEAKKILPNAVYLPWRNLVYWGVSERIMNLLREYSEKIEIASIDEAYLDISDKVRDYREAYNLGLEIKNKILEKEKITVTVGISKNKVFAGYAGTRAKPNGIKVIDDEEVKRLIRELDIADVLGIPYWYAEKLKKLGINKLVDTLSIEFDKLKGMIGEAKAKYLISLARDEYNEPIRTRVRKSIGRTVTMKRNSRNLEEIKPYLFRAIEESYYKLDKRIPKAIHVVAWKSYWDIVSRGRTFPHGISKETAYSESVKLLQKILEEDERKIRRIGVRFSKF

SEQ ID NO: 62 - protein, 340 aa, Sulfolobus solfataricus
MIVLFVDFDYFYAQVEEVLNPSLKGKPVVVCVFSGRFEDSGVVATANYEARKFGVYAGIPIVEAKKILPNAVYLPWRNLVYWGVSERIMNLLREYSEKIEIASIDEAYLDISDKVRDYREAYNLGLEIKNKILEKEKITVTVGISKNKVFAGTAGLMAKPNGIKVIDDEEVKRLIRELDIADVLGIPYWYAEKLKKLGINKLVDTLSIEFDDLRKMIGEAGAVYLISLARDEYNEPIRTRVRKSIGRTVTMKRNSRNLEEIKPYLFRAIEESYYKLDKRIPKAIHVVAWKSYWDIVSRGRTFPHGISKETAYSESVKLLQKILEEDERKIRRIGVRFSKF

SEQ ID NO: 63 - protein, 340 aa, Sulfolobus solfataricus
MIVLFVDFDYFYAQVEEVLNPSLKGKPVVVCVFSGRFEDSGVVATANYEARKFGVYAGIPIVEAKKILPNAVYLPWRNLVYWGVSERIMNLLREYSEKIEIASIDEAYLDISDKVRDYREAYNLGLEIKNKILEKEKITVTVGISKNKVFAGTAGLMAKPNGIKVIDDEEVKRLIRELDIADVLGIPYWYAEKLKKLGINKLVDTLSIEFDFLSTMIGEARARYLISLARDEYNEPIRTRVRKSIGRTVTMKRNSRNLEEIKPYLFRAIEESYYKLDKRIPKAIHVVAWKSYWDIVSRGRTFPHGISKETAYSESVKLLQKILEEDERKIRRIGVRFSKF

SEQ ID NO: 64 - protein, 340 aa, Sulfolobus solfataricus
MIVLFVDFDYFYAQVEEVLNPSLKGKPVVVCVFSGRFEDSGVVATANYEARKFGVYAGIPIVEAKKILPNAVYLPWRNLVYWGVSERIMNLLREYSEKIEIASIDEAYLDISDKVRDYREAYNLGLEIKNKILEKEKITVTVGISKNKVFAGTAGLMAKPNGIKVIDDEEVKRLIRELDIADVLGIPYWYAEKLKKLGINKLVDTLSIEFDKLSEMIGGAGARYLISLARDEYNEPIRTRVRKSIGRTVTMKRNSRNLEEIKPYLFRAIEESYYKLDKRIPKAIHVVAWKSYWDIVSRGRTFPHGISKETAYSESVKLLQKILEEDERKIRRIGVRFSKF

SEQ ID NO: 65 - protein, 340 aa, Sulfolobus solfataricus
MIVLFVDFDYFYAQVEEVLNPSLKGKPVVVCVFSGRFEDSGVVATANYEARKFGVYAGIPIVEAKKILPNAVYLPWRNLVYWGVSERIMNLLREYSEKIEIASIDEAYLDISDKVRDYREAYNLGLEIKNKILEKEKITVTVGISKNKVFAGTAGLMAKPNGIKVIDDEEVKRLIRELDIADVLGIPYWYAEKLKKLGINKLVDTLSIEFDKLKGMIGEAKAKYLISLARDEYNEPIRTRVRKSIGRTVTMKRNSRNLEEIKPYLFRAIEESYYKLDKRIPKAIHVVAWKSYWDIVSRGRTFPHGISKETAYSESVKLLMGVLSVDERKIRRIGVRFSKF

SEQ ID NO: 66 - protein, 340 aa, Sulfolobus solfataricus
MIVLFVDFDYFYAQVEEVLNPSLKGKPVVVCVFSGRFEDSGVVATANYEARKFGVYAGIPIVEAKKILPNAVYLPWRNLVYWGVSERIMNLLREYSEKIEIASIDEAYLDISDKVRDYREAYNLGLEIKNKILEKEKITVTVGISKNKVFAGTAGLMAKPNGIKVIDDEEVKRLIRELDIADVLGIPYWYAEKLKKLGINKLVDTLSIEFDKLKGMIGEAKAKYLISLARDEYNEPIRTRVRKSIGRTVTMKRNSRNLEEIKPYLFRAIEESYYKLDKRIPKAIHVVAWKSYWDIVSRGRTFPHGISKETAYSESVKLLQRILMSDERKIRRIGVRFSKF

SEQ ID NO: 67 - protein, 340 aa, Sulfolobus solfataricus
MIVLFVDFDYFYAQVEEVLNPSLKGKPVVVCVFSGRFEDSGVVATANYEARKFGVYAGIPIVEAKKILPNAVYLPWRNLVYWGVSERIMNLLREYSEKIEIASIDEAYLDISDKVRDYREAYNLGLEIKNKILEKEKITVTVGISKNKVFAGTAGLMAKPNGIKVIDDEEVKRLIRELDIADVLGIPYWYAEKLKKLGINKLVDTLSIEFDKLKGMIGEAKAKYLISLARDEYNEPIRTRVRKSIGRTVTMKRNSRNLEEIKPYLFRAIEESYYKLDKRIPKAIHVVAWKSYWDIVSRGRTFPHGISKETAYSESVKLLKQVLWGDERKIRRIGVRFSKF

SEQ ID NO: 68 - protein, 340 aa, Sulfolobus solfataricus
MIVLFVDFDYFYAQVEEVLNPSLSGLPVVVCVFSGRFEDSGVVATANYEARKFGVYAGIPIVEAKKILPNAVYLPWRNLVYWGVSERIMNLLREYSEKIEIASIDEAYLDISDKVRDYREAYNLGLEIKNKILEKEKITVTVGISKNKVFAGTAGLMAKPNGIKVIDDEEVKRLIRELDIADVLGIPYWYAEKLKKLGINKLVDTLSIEFDKLKGMIGEAKAKYLISLARDEYNEPIRTRVRKSIGRTVTMKRNSRNLEEIKPYLFRAIEESYYKLDKRIPKAIHVVAWKSYWDIVSRGRTFPHGISKETAYSESVKLLQKILEEDERKIRRIGVRFSKF

SEQ ID NO: 69 - protein, 340 aa, Sulfolobus solfataricus
MIVLFVDFDYFYAQVEEVLNPSLKGKPVVVCVFSGRFEDSGVVATANYEARKFGVYAGIPIVEAKKILPNAVYLPWRNLVYWGVSERIMNLLREYSEKIEIASIDEAYLDISDKVRDYREAYNLGLEIKNKILEKEKITVTVGISKNKVFAGTAGLMAKPNGIKVIDDEEVKRLIRELDIADVLGIPYWYAEKLKKLGINKLVDTLSIEFDKLKGMIGEAKAKYLISLARDEYNEPIRTRVRKSIGRTVTMKNNSNNLSQINPYLFRAIEESYYKLDKRIPKAIHVVAWKSYWDIVSRGRTFPHGISKETAYSESVKLLQKILEEDERKIRRIGVRFSKF

SEQ ID NO: 70 - protein, 340 aa, Sulfolobus solfataricus
MIVLFVDFDYFYAQVEEVLNPSLKGKPVVVCVFSGRFEDSGVVATANYEARKFGVYAGIPIVEAKKILPNAVYLPWRNLVYWGVSERIMNLLREYSEKIEIASIDEAYLDISDKVRDYREAYNLGLEIKNKILEKEKITVTVGISKNKVFAGTAGLMAKPNGIKVIDDEEVKRLIRELDIADVLGIPYWYAEKLKKLGINKLVDTLSIEFDKLKGMIGEAKAKYLISLARDEYNEPIRTRVRKSIGRTVTMKRNSRNLEEIKPYLFQAIQESYYKLGNQIPKAIHVVAWKSYWDIVSRGRTFPHGISKETAYSESVKLLQKILEEDERKIRRIGVRFSKF

SEQ ID NO: 71 - protein, 340 aa, Sulfolobus solfataricus
MIVLFVDFDYFYAQVEEVLNPSLKGKPVVVCVFSGRFEDSGVVATANYEARKFGVYAGIPIVEAKKILPNAVYLPWRNLVYWGVSERIMNLLREYSEKIEIASIDEAYLDISDKVRDYREAYNLGLEIKNKILEKEKITVTVGISKNKVFAGTAGLMAKPNGIKVIDDEEVKRLIRELDIADVLGIPYWYAEKLKKLGINKLVDTLSIEFDKLKGMIGEAKAKYLISLARDEYNEPIRTRVRKSIGRTVTMKRNSRNLEEIKPYLFRAIEESYYKLDKRIPSAIHVVAWKSYWDIVSRGSTFPHGISQNTAYSESVKLLQKILEEDERKIRRIGVRFSKF

SEQ ID NO: 72 - protein, 340 aa, Sulfolobus solfataricus
MIVLFVDFDYFYAQVEEVLNPSLKGKPVVVCVFSGRFEDSGVVATANYEARKFGVYAGIPIVEAKKILPNAVYLPWRNLVYWGVSERIMNLLREYSEKIEIASIDEAYLDISDKVRDYREAYNLGLEIKNKILEKEKITVTVGISKNKVFAGTAGLMAKPNGIKVIDDEEVKRLIRELDIADVLGIPYWYAEKLKKLGINKLVDTLSIEFDKLKGMIGEAKAKYLISLARDEYNEPIRTRVRKSIGRTVTMKRNSRNLEEIKPYLFRAIEESYYKLDKRIPKAIHVVAWKSYWDIVSRGRTFPHGISKETAYSQSVQLLQKILKEDKSKIRRIGVRFSKF

SEQ ID NO: 73 - protein, 340 aa, Sulfolobus solfataricus
MIVLFVDFDYFYAQVEEVLNPSLKGKPVVVCVFSGRFEDSGVVATANYEARKFGVYAGIPIVEAKKILPNAVYLPWRNLVYWGVSERIMNLLREYSEKIEIASIDEAYLDISDKVRDYREAYNLGLEIKNKILEKEKITVTVGISKNKVFAGTAGLMAKPNGIKVIDDEEVKRLIRELDIADVLGIPYWYAEKLKKLGINKLVDTLSIEFDKLKGMIGEAKAKYLISLARDEYNEPIRTRVRKSIGRTVTMKRNSRNLEEIKPYLFRAIEESYYKLGNQIPKAIHVVAWKSYWDIVSRGRTFPHGISKDTAYSESVKLLQKILKEDKRKIRRIGVRFSKF

SEQ ID NO: 74 - protein, 340 aa, Sulfolobus solfataricus
MIVLFVDFDYFYAQVEEVLNPSLKGKPVVVCVFSGRFEDSGVVATANYEARKFGVYAGIPIVEAKKILPNAVYLPWRNLVYWGVSERIMNLLREYSEKIEIASIDEAYLDISDKVRDYREAYNLGLEIKNKILEKEKITVTVGISKNKVFAGTAGLMAKPNGIKVIDDEEVKRLIRELDIADVLGIPYWYAEKLKKLGINKLVDTLSIEFDKLRRMIGGARATYLISLARDEYNEPIRTRVRKSIGRTVTMKRNSRNLEEIKPYLFRAIEESYYKLDKRIPKAIHVVAWKSYWDIVSRGRTFPHGISKETAYSESVKLLQKILEEDERKIRRIGVRFSKF

SEQ ID NO: 75 - protein, 340 aa, Sulfolobus solfataricus
MIVLFVDFDYFYAQVEEVLNPSLKGKPVVVCVFSGRFEDSGVVATANYEARKFGVYAGIPIVEAKKILPNAVYLPWRNLVYWGVSERIMNLLREYSEKIEIASIDEAYLDISDKVRDYREAYNLGLEIKNKILEKEKITVTVGISKNKVFAGTAGLMAKPNGIKVIDDEEVKRLIRELDIADVLGIPYWYAEKLKKLGINKLVDTLSIEFDKLAEMIGVAGASYLISLARDEYNEPIRTRVRKSIGRTVTMKRNSRNLEEIKPYLFRAIEESYYKLDKRIPKAIHVVAWKSYWDIVSRGRTFPHGISKETAYSESVKLLQKILEEDERKIRRIGVRFSKF

SEQ ID NO: 76 - protein, 340 aa, Sulfolobus solfataricus
MIVLFVDFDYFYAQVEEVLNPSLKGKPVVVCVFSGRFEDSGVVATANYEARKFGVYAGIPIVEAKKILPNAVYLPWRNLVYWGVSERIMNLLREYSEKIEIASIDEAYLDISDKVRDYREAYNLGLEIKNKILEKEKITVTVGISKNKVFAGTAGLMAKPNGIKVIDDEEVKRLIRELDIADVLGIPYWYAEKLKKLGINKLVDTLSIEFDKLQAMIGLAGARYLISLARDEYNEPIRTRVRKSIGRTVTMKRNSRNLEEIKPYLFRAIEESYYKLDKRIPKAIHVVAWKSYWDIVSRGRTFPHGISKETAYSESVKLLQKILEEDERKIRRIGVRFSKF

SEQ ID NO: 77 - protein, 340 aa, Sulfolobus solfataricus
MIVLFVDFDYFYAQVEEVLNPSLKGKPVVVCVFSGRFEDSGVVATANYEARKFGVYAGIPIVEAKKILPNAVYLPWRNLVYWGVSERIMNLLREYSEKIEIASIDEAYLDISDKVRDYREAYNLGLEIKNKILEKEKITVTVGISKNKVFAGTAGLMAKPNGIKVIDDEEVKRLIRELDIADVLGIPYWYAEKLKKLGINKLVDTLSIEFDKLKGMIGEAKAKYLISLARDEYNEPIRTRVRKSIGRTVTMKRNSRNLEEIKPYLFRAIEESYYKLDKRIPKAIHVVAWKSYWDIVSRGRTFPHGISKETAYSESVKLLIQTLDVDERKIRRIGVRFSKF

SEQ ID NO: 78 - protein, 340 aa, Sulfolobus solfataricus
MIVLFVDFDYFYAQVEEVLNPSLKGKPVVVCVFSGRFEDSGVVATANYEARKFGVYAGIPIVEAKKILPNAVYLPWRNLVYWGVSERIMNLLREYSEKIEIASIDEAYLDISDKVRDYREAYNLGLEIKNKILEKEKITVTVGISKNKVFAGTAGLMAKPNGIKVIDDEEVKRLIRELDIADVLGIPYWYAEKLKKLGINKLVDTLSIEFDKLKGMIGEAKAKYLISLARDEYNEPIRTRVRKSIGRTVTMKRNSRNLEEIKPYLFRAIEESYYKLDKRIPKAIHVVAWKSYWDIVSRGRTFPHGISKETAYSESVKLLTRTLAGDERKIRRIGVRFSKF

SEQ ID NO: 79 - protein, 340 aa, Sulfolobus solfataricus
MIVLFVDFDYFYAQVEEVLNPSLKGKPVVVCVFSGRFEDSGVVATANYEARKFGVYAGIPIVEAKKILPNAVYLPWRNLVYWGVSERIMNLLREYSEKIEIASIDEAYLDISDKVRDYREAYNLGLEIKNKILEKEKITVTVGISKNKVFAGTAGLMAKPNGIKVIDDEEVKRLIRELDIADVLGIPYWYAEKLKKLGINKLVDTLSIEFDKLKGMIGEAKAKYLISLARDEYNEPIRTRVRKSIGRTVTMKRNSRNLEEIKPYLFRAIEESYYKLDKRIPKAIHVVAWKSYWDIVSRGRTFPHGISKETAYSESVKLLNRILRRDERKIRRIGVRFSKF

SEQ ID NO: 80 - protein, 340 aa, Sulfolobus solfataricus
MIVLFVDFDYFYAQVEEVLNPSLKGKPVVVCVFSGRFEDSGVVATANYEARKFGVYAGIPIVEAKKILPNAVYLPWRNLVYWGVSERIMNLLREYSEKIEIASIDEAYLDISDKVRDYREAYNLGLEIKNKILEKEKITVTVGISKNKVFAGTAGLMAKPNGIKVIDDEEVKRLIRELDIADVLGIPYWYAEKLKKLGINKLVDTLSIEFDKLKGMIGEAKAKYLISLARDEYNEPIRTRVRKSIGRTVTMKRNSRNLEEIKPYLFRAIEESYYKLDKRIPKAIHVVAWKSYWDIVSRGRTFPHGISKETAYSESVKLLNSLLRSDERKIRRIGVRFSKF

SEQ ID NO: 81 - protein, 340 aa, Sulfolobus solfataricus
MIVLFVDFDYFYAQVEEVLNPSLKGKPVVVCVFSGRFEDSGVVATANYEARKFGVYAGIPIVEAKKILPNAVYLPWRNLVYWGVSERIMNLLREYSEKIEIASIDEAYLDISDKVRDYREAYNLGLEIKNKILEKEKITVTVGISKNKVFAGTAGLMAKPNGIKVIDDEEVKRLIRELDIADVLGIPYWYAEKLKKLGINKLVDTLSIEFDKLKGMIGEAKAKYLISLARDEYNEPIRTRVRKSIGRTVTMKRNSRNLEEIKPYLFRAIEESYYKLDKRIPKAIHVVAWRSYWSPVTRGGQFPHGISKETAYSESVKLLQKILEEDERKIRRIGVRFSKF

SEQ ID NO: 82 - protein, 340 aa, Sulfolobus solfataricus
MIVLFVDFDYFYAQVEEVLNPSLKGKPVVVCVFSGRFEDSGVVATANYEARKFGVYAGIPIVEAKKILPNAVYLPWRNLVYWGVSERIMNLLREYSEKIEIASIDEAYLDISDKVRDYREAYNLGLEIKNKILEKEKITVTVGISKNKVFAGTAGLMAKPNGIKVIDDEEVKRLIRELDIADVLGIPYWYAEKLKKLGINKLVDTLSIEFTKLAGMIGVAKAKYLISLARDEYNEPIRTRVRKSIGRTVTMKRNSRNLEEIKPYLFRAIEESYYKLDKRIPKAIHVVAWKSYWDIVSRGRTFPHGISKETAYSESVKLLTRCLGVDERKIRRIGVRFSKF

SEQ ID NO: 83 - protein, 340 aa, Sulfolobus solfataricus
MIVLFVDFDYFYAQVEEVLNPSLKGKPVVVCVFSGRFEDSGVVATANYEARKFGVYAGIPIVEAKKILPNAVYLPWRNLVYWGVSERIMNLLREYSEKIEIASIDEAYLDISDKVRDYREAYNLGLEIKNKILEKEKITVTVGISKNKVFAGTAGLMAKPNGIKVIDDEEVKRLIRELDIADVLGIPYWYAEKLKKLGINKLVDTLSIEFTKLAGMIGVAKAKYLISLARDEYNEPIRTRVRKSIGRTVTMKRNSRNLEEIKPYLFRAIEESYYKLDKRIPKAIHVVAWKSYWDIVSRGRTFPHGISKETAYSESVKLLSMCLSADERKIRRIGVRFSKF

SEQ ID NO: 84 - protein, 340 aa, Sulfolobus solfataricus
MIVLFVDFDYFYAQVEEVLNPSLKGKPVVVCVFSGRFEDSGVVATANYEARKFGVYAGIPIVEAKKILPNAVYLPWRNLVYWGVSERIMNLLREYSEKIEIASIDEAYLDISDKVRDYREAYNLGLEIKNKILEKEKITVTVGISKNKVFAGTAGLRAKPNGIKVIDDEMVKGFIRELDIADVLGIPYWYAEKLKKLGINKLVDTLSIEFPKLAGMIGAAKARYLISLARDEYNEPIRTRVRKSIGRTVTMKRNSRNLEEIKPYLFRAIEESYYKLGNQIPKAIHVVAWKSYWQMATLFRHFPHGISKDTAYSESVQLLQQILKKDKRKIRRIGVRFSKF

SEQ ID NO: 85 - protein, 340 aa, Sulfolobus solfataricus
MIVLFVDFDYFYAQVEEVLNPSLKGKPVVVCVFSGRFEDSGVVATANYEARKFGVYAGIPIVEAKKILPNAVYLPWRNLVYWGVSERIMNLLREYSEKIEIASIDEAYLDISDKVRDYREAYNLGLEIKNKILEKEKITVTVGISKNKVFALTAGRMAKPNGIKVIDDEEVKRLIRELDIADVLGIPYWYAEKLKKLGINKLVDTLSIEFDKLKGMIGEAKAKYLISLARDEYNEPIRTRVRKSIGRTVTMKRNSRNLEEIKPYLFRAIEESYYKLDKRIPKAIHVVAWKSYWDAVPRWRFFPHGISKETAYSESVKLLQKILEEDERKIRRIGVRFSKF

SEQ ID NO: 86 - protein, 340 aa, Sulfolobus solfataricus
MIVLFVDFDYFYAQVEEVLNPSLKGKPVVVCVFSGRFEDSGVVATANYEARKFGVYAGIPIVEAKKILPNAVYLPWRNLVYWGVSERIMNLLREYSEKIEIASIDEAYLDISDKVRDYREAYNLGLEIKNKILEKEKITVTVGISKNKVFALTAGRMAKPNGIKVIDDEEVKRLIRELDIADVLGIPYWYAEKLKKLGINKLVDTLSIEFDKLKGMIGEAKAKYLISLARDEYNEPIRTRVRKSIGRTVTMKRNSRNLEEIKPYLFRAIEESYYKLDKRIPKAIHVVAWKSYWDAVPRWRFFPHGISKETAYSESVQLLQQILKKDKRKIRRIGVRFSKF

SEQ ID NO: 87 - protein, 340 aa, Sulfolobus solfataricus
MIVLFVDFDYFYAQVEEVLNPSLKGKPVVVCVFSGRFEDSGVVATANYEARKFGVYAGIPIVEAKKILPNAVYLPWRNLVYWGVSERIMNLLREYSEKIEIASIDEAYLDISDKVRDYREAYNLGLEIKNKILEKEKITVTVGISKNKVFALTAGRMAKPNGIKVIDDEEVKRLIRELDIADVLGIPYWYAEKLKKLGINKLVDTLSIEFDKLKGMIGEAKAKYLISLARDEYNEPIRTRVRKSIGRTVTMKRNSRNLEEIKPYLFRAIEESYYKLDKRIPKAIHVVAWKSYWDCVWRIRWFPHGISKETAYSESVKLLQKILEEDERKIRRIGVRFSKF

SEQ ID NO: 88 - protein, 340 aa, Sulfolobus solfataricus
MIVLFVDFDYFYAQVEEVLNPSLKGKPVVVCVFSGRFEDSGVVATANYEARKFGVYAGIPIVEAKKILPNAVYLPWRNLVYWGVSERIMNLLREYSEKIEIASIDEAYLDISDKVRDYREAYNLGLEIKNKILEKEKITVTVGISKNKVFALTAGRMAKPNGIKVIDDEEVKRLIRELDIADVLGIPYWYAEKLKKLGINKLVDTLSIEFDKLKGMIGEAKAKYLISLARDEYNEPIRTRVRKSIGRTVTMKRNSRNLEEIKPYLFRAIEESYYKLDKRIPKAIHVVAWKSYWDCVWRIRWFPHGISKETAYSESVQLLQQILKKDKRKIRRIGVRFSKF

SEQ ID NO: 89 - protein, 340 aa, Sulfolobus solfataricus
MIVLFVDFDYFYAQVEEVLNPSLKGKPVVVCVFSGRFEDSGVVATANYEARKFGVYAGIPIVEAKKILPNAVYLPWRNLVYWGVSERIMNLLREYSEKIEIASIDEAYLDISDKVRDYREAYNLGLEIKNKILEKEKITVTVGISKNKVFALTAGRMAKPNGIKVIDDEEVKRLIRELDIADVLGIPYWYAEKLKKLGINKLVDTLSIEFDKLKGMIGEAKAKYLISLARDEYNEPIRTRVRKSIGRTVTMKRNSRNLEEIKPYLFRAIEESYYKLDKRIPKAIHVVAWKSYWDYVWRWRVFPHGISKETAYSESVKLLQKILEEDERKIRRIGVRFSKF

SEQ ID NO: 90 - protein, 340 aa, Sulfolobus solfataricus
MIVLFVDFDYFYAQVEEVLNPSLKGKPVVVCVFSGRFEDSGVVATANYEARKFGVYPGIPIVEAKKILPNAVYLPWRNLVYWGVSERIMNLLREYSEKIEIASIDEAYLDISDKVRDYREAYNLGLEIKNKILEKEKITVTVGISKNKVFALTAGRMAKPNGIKVIDDEEVKRLIRELDIADVLGIPYWYAEKLKKLGINKLVDTLSIEFDKLKGMIGEAKAKYLISLARDEYNEPIRTRVRKSIGRTVTMKRNSRNLEEIKPYLFRAIEESYYKLDKRIPKAIHVVAWKSYWDYVHRLRRFPHGISKETAYSESVKLLQKILEEDERKIRRIGVRFSKF

SEQ ID NO: 91 - protein, 340 aa, Sulfolobus solfataricus
MIVLFVDFDYFYAQVEEVLNPSLKGKPVVVCVFSGRFEDSGVVATANYEARKFGVYPGIPIVEAKKILPNAVYLPWRNLVYWGVSERIMNLLREYSEKIEIASIDEAYLDISDKVRDYREAYNLGLEIKNKILEKEKITVTVGISKNKVFALTAGRMAKPNGIKVIDDEEVKRLIRELDIADVLGIPYWYAEKLKKLGINKLVDTLSIEFDKLKGMIGEAKAKYLISLARDEYNEPIRTRVRKSIGRTVTMKRNSRNLEEIKPYLFRAIEESYYKLDKRIPKAIHVVAWKSYWDYVHRLRRFPHGISKETAYSESVQLLQQILKKDKRKIRRIGVRFSKF

SEQ ID NO: 92 - protein, 340 aa, Sulfolobus solfataricus
MIVLFVDFDYFYAQVEEVLNPSLKGKPVVVCVFSGRFEDSGVVATANYEARKFGVYPGIPIVEAKKILPNAVYLPWRNLVYWGVSERIMNLLREYSEKIEIASIDEAYLDISDKVRDYREAYNLGLEIKNKILEKEKITVTVGISKNKVFALTAGRMAKPNGIKVIDDEEVKRLIRELDIADVLGIPYWYARKLKLLGINKLVDTLSIEFDKLKGMIGEAKAKYLISLARDEYNEPIRTRVWKSIGRTVTMKRNSRNLEEIKPYLFRAIEESYYKLDKRIPGAIHVVAWKSYWDYVHRLRRFPHGISKETAYSESVKLLQKILKEDKRKIRRIGVRFSKF

SEQ ID NO: 93 - protein, 340 aa, Sulfolobus solfataricus
MIVLFVDFDYFYAQVEEVLNPSLKGKPVVVCVFSGRFEDSGVVATANYEARKFGVYPGIPIVEAKKILPNAVYLPWRNLVYWGVSERIMNLLREYSEKIEIASIDEAYLDISDKVRDYREAYNLGLEIKNKILEKEKITVTVGISKNKVFALTAGRMAKPNGIKVIDDEEVKRLIRELDIADVLGIPYWYARKLKLLGINKLVDTLSIEFDKLKGMIGEAKAKYLISLARDEYNEPIRTRVWKSIGRTVTMKRNSRNLEEIKPYLFRAIEESYYKLDKRIPGAIHVVAWKSYWQMATLFRHFPHGISKETAYSESVQLLQQILKKDKRKIRRIGVRFSKF

SEQ ID NO: 94 - protein, 340 aa, Sulfolobus solfataricus
MIVLFVDFDYFYAQVEEVLNPSLKGKPVVVCVFSGRFEDSGVVATANYEARKFGVYPGIPIVEAKKILPNAVYLPWRNLVYWGVSERIMNLLREYSEKIEIASIDEAYLDISDKVRDYREAYNLGLEIKNKILEKEKITVTVGISKNKVFALTAGRMAKPNGIKVIDDEEVKRLIRELDIADVLGIPYWYARKLKLLGINKLVDTLSIEFDKLKGMIGEAKAKYLISLARDEYNEPIRTRVWKSIGRTVTMKRNSRNLEEIKPYLFRAIEESYYKLDKRIPGAIHVVAWKSYWQMATLFRHFPHGISKETAYSESVKLLQKILKEDKRKIRRIGVRFSKF

SEQ ID NO: 95 - protein, 340 aa, Sulfolobus solfataricus
MIVLFVDFDYFYAQVEEVLNPSLKGKPVVVCVFSGRFEDSGVVATANYEARKFGVYAGIPIVEAKKILPNAVYLPWRNLVYWGVSERIMNLLREYSEKIEIASIDEAYLDISDKVRDYREAYNLGLEIKNKILEKEKITVTVGISKNKVFALTAGRMAKPNGIKVIDDEEVKRLIRELDIADVLGIPYWYAEKLKKLGINKLVDTLSIEFDKLKGMIGEAKAKYLISLARDEYNEPIRTRVRKSIGRTVTMKRNSRNLEEIKPYLFRAIEESYYKLDKRIPKAIHVVAWKSYWNSQYRWSWFPHGISKETAYSESVQLLQQILKKDKRKIRRIGVRFSKF

SEQ ID NO: 96 - protein, 340 aa, Sulfolobus solfataricus
MIVLFVDFDYFYAQVEEVLNPSLKGKPVVVCVFSGRFEDSGVVATANYEARKFGVYAGIPIVEAKKILPNAVYLPWRNLVYWGVSERIMNLLREYSEKIEIASIDEAYLDISDKVRDYREAYNLGLEIKNKILEKEKITVTVGISKNKVFAAKAAIMAKPNGIKVIDDEEVKRLIRELDIADLLGIPYWYAEKLKKLGINKLVDTLSIEFDKLKGMIGEAKAKYLISLARDEYNEPIRTRVRKSIGRTVTMKRNSRNLEEIKPYLFRAIEESYYKLDKRIPKAIHVVAWKSYWQMATLFRHFPHGISKETAYSESVKLLQKILEEDERKIRRIGVRFSKF

SEQ ID NO: 97 - protein, 340 aa, Sulfolobus solfataricus
MIVLFVDFDYFYAQVEEVLNPSLKGKPVVVCVFSGRFEDSGVVATANYEARKFGVYAGIPIVEAKKILPNAVYLPWRNLVYWGVSERIMNLLREYSEKIEIASIDEAYLDISDKVRDYREAYNLGLEIKNKILEKEKITVTVGISKNKVFAQRAGAMAKPNGIKVIDDEEVKRLIRELDIADVLGIPYWYAEKLKKLGINKLVDTLSIEFDKLKGMIGEAKAKYLISLARDEYNEPIRTRVRKSIGRTVTMKRNSRNLEEIKPYLFRAIEESYYKLDKRIPKAIHVVAWKSYWQMATLFRHFPHGISKETAYSESVKLLQKILEEDERKIRRIGVRFSKF

SEQ ID NO: 98 - protein, 340 aa, Sulfolobus solfataricus
MIVLFVDFDYFYAQVEEVLNPSLKGKPVVVCVFSGRFEDSGVVATANYEARKFGVYAGIPIVEAKKILPNAVYLPWRNLVYWGVSERIMNLLREYSEKIEIASIDEAYLDISDKVRDYREAYNLGLEIKNKILEKEKITVTVGISKNKVFAVYACGMAKPNGIKVIDDEEVKRLIRELDIADVLGIPYWYAEKLKKLGINKLVDTLSIEFDKLKGMIGEAKAKYLISLARDEYNEPIRTRVRKSIGRTVTMKRNSRNLEEIKPYLFRAIEESYYKLDKRIPKAIHVVAWKSYWQMATLFRHFPHGISKETAYSESVKLLQKILEEDERKIRRIGVRFSKF

SEQ ID NO: 99 - protein, 340 aa, Sulfolobus solfataricus
MIVLFVDFDYFYAQVEEVLNPSLKGKPVVVCVFSGRFEDSGVVATANYEARKFGVYAGIPIVEAKKILPNAVYLPWRNLVYWGVSERIMNLLREYSEKIEIASIDEAYLDISDKVRDYREAYNLGLEIKNKILEKEKITVTVGISKNKVFALTAGRMAKPNGIKVIDDEMVKGFIRELDIADVLGIPYWYAEKLKKLGINKLVDTLSIEFDKLKGMIGEAKAKYLISLARDEYNEPIRTRVRKSIGRTVTMKRNSRNLEEIKPYLFRAIEESYYKLDKRIPKAIHVVAWKSYWQMATLFRHFPHGISKETAYSESVKLLQKILEEDERKIRRIGVRFSKF

SEQ ID NO: 100 - protein, 340 aa, Sulfolobus solfataricus
MIVLFVDFDYFYAQVEEVLNPSLKGKPVVVCVFSGRFEDSGVVATANYEARKFGVYAGIPIVEAKKILPNAVYLPWRNLVYWGVSERIMNLLREYSEKIEIASIDEAYLDISDKVRDYREAYNLGLEIKNKILEKEKITVTVGISKNKVFALTAGRMAKPNGIKVIDDEEVKRLIRELDIADVLGIPYWYAEKLKKLGINKLVDTLSIEFPKLVGMIGAAKATYLISLARDEYNEPIRTRVRKSIGRTVTMKRNSRNLEEIKPYLFRAIEESYYKLDKRIPKAIHVVAWKSYWQMATLFRHFPHGISKETAYSESVKLLQKILEEDERKIRRIGVRFSKF

SEQ ID NO: 101 - protein, 340 aa, Sulfolobus solfataricus
MIVLFVDFDYFYAQVEEVLNPSLKGKPVVVCVFSGRFEDSGVVATANYEARKFGVYAGIPIVEAKKILPNAVYLPWRNLVYWGVSERIMNLLREYSEKIEIASIDEAYLDISDKVRDYREAYNLGLEIKNKILEKEKITVTVGISKNKVFAAKAAIMAKPNGIKVIDDEEVKRLIRELDIADVLGIPYWYAEKLKKLGINKLVDTLSIEFDKLKGMIGEAKAKYLISLARDEYNEPIRTRVRKSIGRTVTMKRNSRNLEEIKPYLFRAIEESYYKLDKRIPKAIHVVAWKSYWDIVSRGRTFPHGISKETAYSESVQLLQQILKKDKRKIRRIGVRFSKF

SEQ ID NO: 102 - protein, 340 aa, Sulfolobus solfataricus
MIVLFVDFDYFYAQVEEVLNPSLKGKPVVVCVFSGRFEDSGVVATANYEARKFGVYAGIPIVEAKKILPNAVYLPWRNLVYWGVSERIMNLLREYSEKIEIASIDEAYLDISDKVRDYREAYNLGLEIKNKILEKEKITVTVGISKNKVFAQRAGAMAKPNGIKVIDDEEVKRLIRELDIADVLGIPYWYAEKLKKLGINKLVDTLSIEFDKLKGMIGEAKAKYLISLARDEYNEPIRTRVRKSIGRTVTMKRNSRNLEEIKPYLFRAIEESYYKLDKRIPKAIHVVAWKSYWDIVSRGRTFPHGISKETAYSESVQLLQQILKKDKRKIRRIGVRFSKF

SEQ ID NO: 103 - protein, 340 aa, Sulfolobus solfataricus
MIVLFVDFDYFYAQVEEVLNPSLKGKPVVVCVFSGRFEDSGVVATANYEARKFGVYPGIPIVEAKKILPNAVYLPWRNLVYWGVSERIMNLLREYSEKIEIASIDEAYLDISDKVRDYREAYNLGLEIKNKILEKEKITVTVGISKNKVFAQRAGAMAKPNGIKVIDDEEVKRLIRELDIADVLGIPYWYAEKLKKLGINKLVDTLSIEFDKLKGMIGEAKAKYLISLARDEYNEPIRTRVRKSIGRTVTMKRNSRNLEEIKPYLFRAIEESYYKLDKRIPKAIHVVAWKSYWDYVHRLRRFPHGISKETAYSESVQLLQQILKKDKRKIRRIGVRFSKF

SEQ ID NO: 104 - protein, 340 aa, Sulfolobus solfataricus
MIVLFVDFDYFYAQVEEVLNPSLKGKPVVVCVFSGRFEDSGVVATANYEARKFGVYAGIPIVEAKKILPNAVYLPWRNLVYWGVSERIMNLLREYSEKIEIASIDEAYLDISDKVRDYREAYNLGLEIKNKILEKEKITVTVGISKNKVFAQRAGAMAKPNGIKVIDDEEVKRLIRELDIADVLGIPYWYAEKLKKLGINKLVDTLSIEFDKLKGMIGEAKAKYLISLARDEYNEPIRTRVRKSIGRTVTMKRNSRNLEEIKPYLFRAIEESYYKLDKRIPKAIHVVAWKSYWQMATLFRHFPHGISKETAYSESVQLLQQILKKDKRKIRRIGVRFSKF

SEQ ID NO: 105 - protein, 340 aa, Sulfolobus solfataricus
MIVLFVDFDYFYAQVEEVLNPSLKGKPVVVCVFSGRFEDSGVVATANYEARKFGVYAGIPIVEAKKILPNAVYLPWRNLVYWGVSERIMNLLREYSEKIEIASIDEAYLDISDKVRDYREAYNLGLEIKNKILEKEKITVTVGISKNKVFALTAGRMAKPNGIKVIDDEEVKRLIRELDIADVLGIPYWYAEKLKKLGINKLVDTLSIEFPKLAGMIGAAKARYLISLARDEYNEPIRTRVRKSIGRTVTMKRNSRNLEEIKPYLFRAIEESYYKLDKRIPKAIHVVAWKSYWDIVSRGRTFPHGISKETAYSESVQLLQQILKKDKRKIRRIGVRFSKF

SEQ ID NO: 106 - protein, 340 aa, Sulfolobus solfataricus
MIVLFVDFDYFYAQVEEVLNPSLKGKPVVVCVFSGRFEDSGVVATANYEARKFGVYAGIPIVEAKKILPNAVYLPWRNLVYWGVSERIMNLLREYSEKIEIASIDEAYLDISDKVRDYREAYNLGLEIKNKILEKEKITVTVGISKNKVFALTAGRMAKPNGIKVIDDEMVKGFIRELDIADVLGIPYWYAEKLKKLGINKLVDTLSIEFDKLKGMIGEAKAKYLISLARDEYNEPIRTRVRKSIGRTVTMKRNSRNPEEIKPYLFRAIEESYYKLDKRIPKAIHVVAWKSYWQMATLFRHFPHGISKETAYSESVKLLQKILEEDERKIRRIGVRFSKF